European Patent Specification EP 3 383 888 B9, published October 4, 2023. Title: NEW PEPTIDES HAVING ANTIMICROBIAL ACTIVITY AND NEW ENZYME CAPABLE OF CONVERTING L-CONFIGURED RESIDUE IN D-CONFIGURED AMINO ACID IN A PEPTIDE. Applicant: INRA. The sequence listing filed with the application follows.

SEQUENCE LISTING (73 sequences)

SEQ ID NO: 1 - protein, 49 aa, Bacillus subtilis
MKKEITNNETVKNLEFKGLLDESQKLAKVNDLWYFVKSKENRWILGSGH

SEQ ID NO: 2 - protein, 49 aa, Bacillus subtilis
MKKENTNNETVKNLEFKGLLDESQKLAKVNDLWYFVKSKENRWILGSGH

SEQ ID NO: 3 - protein, 49 aa, Bacillus sp
MKKENTNNETVKNLEFKGLLDESQKLAKVNDLWYFVKSQENRWILGSGH

SEQ ID NO: 4 - protein, 49 aa, Bacillus subtilis
MKKENTNNEPVKNLEFKGLLDESQKLAKVNDLWYFVKSKENRWILGSGH

SEQ ID NO: 5 - protein, 49 aa, Bacillus coagulans
MSKENTQNSNVKNLEFKSLVEESQKLAKVNDLWYFVKSKGNRWIVGSGH

SEQ ID NO: 6 - protein, 54 aa, Staphylococcus pseudintermedius
MKKEINSYKSTKENTMKDLEFKKLVNDSEKLAKVNDLWYFVKSQSNRWIVGSGH

SEQ ID NO: 7 - protein, 54 aa, Staphylococcus equorum
MKENLKVEKQNKKEVMKDLEFKTLINDSQKLAKVNDLWYFVKSKQNRWVVGSGH

SEQ ID NO: 8 - protein, 62 aa, Staphylococcus condimenti
MKGKGDIKKNKDVQIQKKDKKDAMKNLEFKNLVNDSEKLAKVNDLWYFVKSKSHRWIVGSGH

SEQ ID NO: 9 - protein, 54 aa, Staphylococcus epidermidis
MNKDLHNQKNNKQDVMKDLEFKNLVNNSEKLAKVNDLWYFVKSKANRWVVGSGH

SEQ ID NO: 10 - protein, 42 aa, Paenibacillus sp
MKKLEIKELISKSEKLAKVNDLWYFVRSGEGAWIVGSGGGSK

SEQ ID NO: 11 - protein, 39 aa, Enterococcus caccae
MKELEMKELVEKSEKLAKVNDLWYFVKSSSGAWIAGSGR

SEQ ID NO: 12 - protein, 39 aa, Enterococcus faecalis
MKELEMKELVEKSEKLAKINDLWYFVKSKGGAWIAGSGK

SEQ ID NO: 13 - protein, 49 aa, Enterococcus faecalis
MWNNYKGDIIMKELEMKELVEKSEKLAKINDLWYFVKSKGGAWIAGSGK

SEQ ID NO: 14 - protein, 54 aa, Streptococcus agalactiae
MTIEIKNIQREVKPILNDMSFAKVLTKKNKLDNVNDLWYFVRNSKNRWVAGSAH

SEQ ID NO: 15 - protein, 52 aa, Streptococcus agalactiae
MKQKNIQREVKPILNDMSFAKVLTKKNELDNVNDLWYFVRSSKNRWVAGSAH

SEQ ID NO: 16 - protein, 36 aa, Streptococcus
MSFAKVLTKKNKLDNVNDLWYFVRNSKNRWVAGSAH

SEQ ID NO: 17 - protein, 49 aa, Enterococcus faecalis
MCNNYKGDIIMKELEMKELVEKSEKLAKINDLWYFVKSKGGAWIAGSGK

SEQ ID NO: 18 - protein, 44 aa, Enterococcus faecalis
MCNNYKGDIIMKELVEKSEKLAKINDLWYFVKSKGGAWIAGSGK

SEQ ID NO: 19 - protein, 40 aa, Bifidobacterium bohemicum
MEKSSEILNSLQANENVIDLEDQDDLWYFIKGGGNWIMGS

SEQ ID NO: 20 - protein, 32 aa, artificial sequence
  YyFd18-49
GLLDESQKLAKVNDLWYFVKSKENRWILGSGH

SEQ ID NO: 21 - protein, 7 aa, artificial sequence
  motif
  MISC_FEATURE (1)..(1): X is D or N
  MISC_FEATURE (7)..(7): X is I, V or A
XDLWYFX

SEQ ID NO: 22 - protein, 5 aa, artificial sequence
  motif
  MISC_FEATURE (2)..(2): X is I or V
  MISC_FEATURE (3)..(3): X is any amino acid
WXXGS

SEQ ID NO: 23 - protein, 11 aa, artificial sequence
  motif
  MISC_FEATURE (2)..(2): X is A, D or E
  MISC_FEATURE (3)..(3): X is K, N or D
  MISC_FEATURE (4)..(4): X is V, I or Q
  MISC_FEATURE (11)..(11): X is V or I
LXXXNDLWYFX

SEQ ID NO: 24 - protein, 11 aa, artificial sequence
  motif
LAKVNDLWYFV

SEQ ID NO: 25 - protein, 319 aa, Bacillus subtilis
MYNKTVSINLDSRCNASCDHCCFSSSPTSTTRMEKEYIRELVTEFAKNKTIQVISFTGGEVFLDYKFLKELMEIIKPYEKQITLISNGFWGLSKKKVQEYFHDMNSLNVIALTISYDEYHAPFVKSSSIKNILEHSRKYPDIDISLNMAVTKDKMSNHILEELGDSILGVKITKFPMISVGAAKTRIKQENIHKFYSLEDEDSLHCPGYDIVYHHDGEIYPCCSPAIFETKITLREEYNQSFERTVEKLNSNLLLFILRKEGFKWFLNILKENNKIEEFDIPYEFSSICGVCGSLFNSAEKINYFYPYMEKYYNENFKV

SEQ ID NO: 26 - protein, 319 aa, Bacillus subtilis
MYNKTVSINLDSRCNASCDHCCFSSSPSSTTRMEKEYIRELVTEFAKNKTIQVISFTGGEVFLDYKFLKELMEIIKPYEKQITLISNGFWGLSKKKVQEYFHDMNSLNVIALTISYDEYHAPFVKSSSIKNILEHSRKYPDIDISLNMAVTKDKMSNHILEELGDSILGVKITKFPMISVGAAKTRIKQENIHKFYSLEDEDSLHCPGYDIVYHHDGEIYPCCSPAIFETKITLREEYNQSFERTVEKLNSNLLLFILRKEGFKWFLNILKENNKIEEFDIPYEFSSICGVCGSLFNSAEKINYFYPYMEKYYNENFKV

SEQ ID NO: 27 - protein, 319 aa, Bacillus subtilis
MYNKTVSINLDSRCNASCDHCCFSSSPTSTTRMEKEYIRELVTEFAKNKTIQVISFTGGEVFLDYKFLKELMEIIKPYEKQITLISNGFWGLSKKKVQEYFHDMSSLNVIALTISYDEYHAPFVKSSSIKNILEHSRKYPDIDISLNMAVTKDKMSNHILEELGDSILGVKITKFPMISVGAAKTRIKQENIHKFYSLEDEDSLHCPGYDIVYHHDGEIYPCCSPAIFETKITLREEYNQSFERTVEKLNSNLLLFILRKEGFKWFLNILKENNKIEEFDIPYEFSSICGVCGSLFNSAEKINYFYPYMEKYYNENFKV

SEQ ID NO: 28 - protein, 319 aa, Bacillus subtilis
MYNKTVSINLDSRCNASCDHCCFSSSPTSTIRMEKEYIRELVTEFAKNKTIQVISFTGGEVFLDYKFLKELMEIIKPYEKQITLISNGFWGLSKKKVQEYFHDMNSLNVIALTISYDEYHAPFVKSSSIKNILEHSRKYPDIDISLNMAVTKDKMSNHILEELGDSILGVKITKFPMISVGAAKTRIKQENIHKFYSLEDEDSLHCPGYDIVYHHDGEIYPCCSPAIFETKITLREEYNQSFERTVEKLNSNLLLFILRKEGFKWFLNILKENNKIEEFDIPYEFSSICGVCGSLFNSAEKINYFYPYMEKYYNENFKV

SEQ ID NO: 29 - protein, 319 aa, Bacillus subtilis
MYNKTVSINLDSRCNASCDHCCFSSSPTSTTRMEKEYIRELVTEFAKNKTIQVISFTGGEVFLDYKFLKELMEIIKPYEKQITLISNGFWGMSKKRVQEYFHDMNSLNVIALTISYDEYHAPFVKSSSIKNILEHSRKYPDIDISLNMAVTKDKMSNHILEELGDSILGVKITKFPMISVGAAKTRIKQENIHKFYSLEDEDSLHCPGYDIVYHHDGEIYPCCSPAIFETKITLREEYSQSFERTVEKLNSNLLLFILRKEGFKWFLNILKENNKIEEFDIPYEFSSICGVCGSLFNSAEKINYFYPYMEKYYNENFKV

SEQ ID NO: 30 - protein, 319 aa, Bacillus sp
MYNKTVSINLDSRCNASCDHCCFSSSPSSTTMMEKEYIRELVTEFAKNKTIQVISFTGGEVFLDYKFLKELMEIIKPYEKQITLISNGFWGLSKKKVQEYFHDMNSLNVIALTISYDEYHAPFVKSSSIKNILEHSRKYPDIDISLNMAVTKDKMSNHILEELGDSILGVKITKFPMISVGAAKTRIKQENIHKFYSLEDEDSLHCPGYDIVYHHDGEIYPCCSPAIFETKITLREEYNQSFERTVEKLNSNLLLFILRKEGFKWFLNILKENNKIEEFDIPYEFSSICGVCGSLFNSAEKINYFYPYMEKYYNENFKV

SEQ ID NO: 31 - protein, 320 aa, Salinibacillus aidingensis
MYNKTVSINLDSRCNASCDHCCFSSSPTSTTRMEKEYIRELVTEFAKNKTIQVISFTGGEVFLDYKFLKELMEIIKPYEKQITLISNGFWGISKKKVQEYFHDMNSLNVIALTISYDEYHAPFVKPSSVKRIFEHSRKYRGSIDISLNMAVTKDKMSNHILEELGDSILGVKITKFPMISVGAAKNRIKQENIHKFYSLEDEDSLHCPGYDIVYHHDGEIYPCCSPAIFETKITLREEYNQSFERTVEKLNSNLLLFILRKEGFKWFLNILKENNKIEEFDIPYEFSSICGVCGSLFNSAEKINYFYPYMEKYYNENFKV

SEQ ID NO: 32 - protein, 319 aa, Bacillus subtilis
MYDKTVSINLDSKCNASCDHCCFSSSPTSTIKMEKDYIRDLVTEFAKNKTIQVISFTGGEIFLDYIFLKELMEIIKPYEKQITLISNGFWGVSRKRVQEYFYDMNSLNVVALTISYDEYHAPFVKSSSIKNILEHSRKYPDIDISLNMAVTKDKMSNHILEELGDSILGVKITKFPMISVGAARTRIRQENIHKFYNLDDEDSLYCPGYEIVYHHDGEIYPCCSPAIFETKITLREEYNQNFERTVEKLNSNLLLFILRKEGFKWFLDILKENNKIEEFDIPYEFSSICGVCGSLFNSAEKINYFYPHMEKYYYENFEV

SEQ ID NO: 33 - protein, 319 aa, Bacillus tequilensis
MYDKTVSINLDSKCNASCDHCCFSSSPTSTIKMEKDYIRDLVTEFAKNKTIQVISFTGGEIFLDYIFLKELMEIIKPYEKQITLISNGFWGVSRKRVQEYFYDMNSLNVVALTISYDEYHAPFVKSSSIKNILEHSRKYPDIDISLNMAVTKDKMSNHILEDLGDSILGVKITKFPMISVGAARTRIRPENIHKFHNLDDDDSLYCPGYEIVYHHDGEIYPCCSPAIFETKITLREEYNQNFERTVEKLNSNLLLFILRKEGFKWFLDILKENNKIEEFDIPYEFSSICGVCGSLFNSAEKINYFYPHMEKYYYENFEV

SEQ ID NO: 34 - protein, 320 aa, Bacillus
MYDKTVSINLDSKCNAQCDHCCFSSSPTSTIKMEKDYIRKLVTEFAENKTIQVISFTGGEVFLDYTFLKELMEIIKPYEKQITLISNGFWGISKKKVQEYFHDMNTLNVVALTISYDEYHAPFVKPSSIKRIFEHSRKYRGSIDISLNMAVTKDKMSNHILEELGDSILGVKITKFPMISVGAAKSRIKQENIHKFYSLEDEDSLQCPGYDIVYHHDGEIYPCCSPAIFETKITLREDYNQNFERTVEKLKSNLLLFILRKEGFKWFLDILKDNNKIEEFDIPYEFSSICGVCGSLFNSVEKINYFYPYMEKYYHENFEV

SEQ ID NO: 35 - protein, 327 aa, Bacillus coagulans
MYNKTVAINLDSKCNASCDHCCFSSSPTSEVKMEKDYIRNLVNEFARSKTIEVISFTGGEIFLDYKFLKELMEIIKPYKKQITLISNGFWGGSQNKVEEYFKDMNSLNVVALTISYDEYHAPFVKLSSVKRIFEHSRKYPDIDVSLNMAVTKDKMSNRILEELGDSILGIKITKFPLIPVGAAKNRISQENIHKFYNLDDEDSLQCPGYEIVYHHDGEIYPCCSPAIFETKITLREEYSQTYERTVEKLQSNLLLFIIRKEGFKWFLNILKENKKIEEFGIPYEFSSICSLCVSLFNSEDKINYFHNFMEDYYYANYGNKDHETAKI

SEQ ID NO: 36 - protein, 319 aa, Staphylococcus equorum
MYINSVSINLDSKCNAACDHCCFSCSPQSTIKMEDSYIRKQVLEFSKNPNIKVISFTGGEIFLNYQFLEELLKITKFYNKKITLISNGFWGASRRLLRKYFEDFQKYNVVALTISYDEYHSPYVKIKSIKNIFDYRMKYPEIEVSLNMAVTKEKMSDNILRELGSSVLGIKITKFPMITVGAAKKNIAKENIHNFYNVEKDKSILYCPGYELVYHHDGEIYPCCSPAIFETSITLRESENQTFERTIEKLNSNLLLYIIRKEGFNWFIKILKNNNLMDSFEIPEDFPSVCSVCGSLFNSEEKIEFFKPYMEKYYENFEI

SEQ ID NO: 37 - protein, 320 aa, Staphylococcus pseudintermedius
MYDKSVSINLTSKCNATCDHCCFSCSPKSTIKMEDFYIRETVLEFAKDSNVEVISFTGGEIFLNYEFLEELLKITKNYNKKVTLISNGFWGNSRKLLEKYFSDFYKYNVVALTISYDEYHSPFVKLKSIKNIFEYRMKYPEIQVSLNMAVTKDKMSDNILRELGSSILGAKITKFPMISVGAAKDKISKENIHNFYNINKDREVLYCPGFEIVYHHDGEIYPCCSPAIFETPITLRENKNQTLTRTVEKLNSNLLLYIIRKEGFNWFLDILREENMLHQFDIPTDFPSVCSICGSLFSTEEKIKFFKPFMEAYYYETIEV

SEQ ID NO: 38 - protein, 320 aa, Staphylococcus epidermidis
MYGKSVSINLNSKCNAMCDHCCFSCSPKSTIKMKDSYIKDTVLEFSKNPNIEIISFTGGEIFLNYKFLEELLIITKSYNKKVTLISNGFWGSSRKLLRKFFDDFKKYNVIALTISYDEYHEPFIKLKSVKNIFEYRMKYPEIEVSLNMAVTKDKMSDNILSELGSSILGIKITKFPMITVGSAKNKISKNNIHNFYNIEKDKNLLFCPGYEIVYHHDGEIYPCCSPAIFETKISLREDKYQTLERTIEKLNSNLLLYIVRKEGFNWFLDIVREQDLLNEFEIPKDFPSVCSICGNLFNTEEKINFFKPYMKEYYYETIKV

SEQ ID NO: 39 - protein, 315 aa, Paenibacillus sp
MYNNAVINLGAKCNAACAHCCFSCSPASTQSMEPNYIRQLAHELAENKKVNLISFTGGEIFLNYPFLQELLEIIKPHQKRITLISNGFWGMSRKKTEQYFNDMEYYNVTNLTISYDEFHEPYVKADAIKNILECSRDFSNTSVALNMAVTKSKMSNRILEYMGESLLGIRVTKFPLMPVGEAKHEEPDSFQHIYKLSNERSLHCPGFEVVYHFDGQIYPCCSPAVFDTKLHLRESMDQTFDRTIEKLNANLLFYIMRKEGFKWFIDIVQSNPEFNHIKIPEQFSSICNICNILFKTEENIDLLTPYMMNYYENMV

SEQ ID NO: 40 - protein, 335 aa, Paenibacillus sp
MYKITLLHLTSFKNGRKEMFMYNNAVINLGAKCNAACAHCCFSCSPASTQSMEPNYIRQLAHELAENKKVNLISFTGGEIFLNYPFLQELLEIIKPHQKRITLISNGFWGMSRKKTEQYFNDMEYYNVTNLTISYDEFHEPYVKADAIKNILECSRDFSNTSVALNMAVTKSKMSNRILEYMGESLLGIRVTKFPLMPVGEAKHEEPDSFQHIYKLSNERSLHCPGFEVVYHFDGQIYPCCSPAVFDTKLHLRESMDQTFDRTIEKLNANLLFYIMRKEGFKWFIDIVQSNPEFNHIKIPEQFSSICNICNILFKTEENIDLLTPYMMNYYENMV

SEQ ID NO: 41 - protein, 335 aa, Enterococcus caccae
MYEITLLHLTSFKNGRKEMFMYNNAVINLGAKCNAACAHCCFSCSPASTQSMEPNYIRQLAHELAENKKVNLISFTGGEIFLNYPFLQELLEIIKPHQKRITLISNGFWGMSRKKTEQYFNDMEYYNVTNLTISYDEFHEPYVKADAIKNILECSRDFSNTSVALNMAVTKSKMSNRILEYMGESLLGIRVTKFPLMPVGEAKHEEPDSFQHIYKLSNERSLHCPGFEVVYHFDGQIYPCCSPAVFDTKLHLRESMDQTFDRTIEKLNANLLFYIMRKEGFKWFIDIVQSNPEFNHIKIPEQFSSICNICNILFKTEENIDLLTPYMMNYYENMV

SEQ ID NO: 42 - protein, 315 aa, Enterococcus faecalis
MYESVVINLGARCNATCEHCCFSCSPSKKTSMEKSEIIELVKSFSNNLKIKVISFTGGEIFLNYSFLKELLEIVHSCGKKSTLISNGFWGANVEKVKIYFKDMKELGVTNLSISHDDFHAKFVKTDCIKNILEESRKYPSIRVVVNIAVSKSNMGNKVIEELDEAALGIPLTKYPLIAVGEAENMADSEFQKIYSIDNLEQLECPGYEPVYHFDGNVYPCCSPAVFDTALILNDRACQSFDKTIEKMNANLLLYIMRKEGFRWFIEIVMSNQEFSHIQIEEHFSSICTICRQLFKSEENIKLFTPYMREYYEQML

SEQ ID NO: 43 - protein, 318 aa, Enterococcus faecalis
MNLLYESVVVNLGARCNASCEHCCFSCSPTKKEALDKNEVINLVENFSNNPKIKTISFTGGEIFLNYPFLYSLLKIVNSSGKISTLISNGFWGREIETVKKYFLDMNRMGVTNLSISHDDFHSKFIKTDYIRNILIESRKYPDIQITVNIAVSKNSTGDKIIHDLGEAILGIPVTKFPLIPVGEAKNINDDEFQNIYSLSHPNQLKCPGFEPVYHFNGNVYPCCSPAIFDTALILNDELYQDFDKTITKMNSNLLLYIMRREGFSWFINIVSNNNEFSHIKINKEFSSICSICRQLFKTENNIKLLTPYMRKYYEQML

SEQ ID NO: 44 - protein, 315 aa, Enterococcus faecalis
MYDSVVVNLGARCNASCEHCCFSCSPTKKEALDKKEVINLVENFSNNPKIKTISFTGGEIFLNYPFLYNLLKIVNSSGKISTLISNGFWGREIETVKKYFLDMNRMGVTNLSISHDDFHSKFIKTDYIRNILIESRKYPDIQITVNIAVSKNSTGDKIIHDLGEAILGIPVTKFPLIPVGEAKNINDDEFQNIYSLSHPNQLKCPGFEPVYHFNGNVYPCCSPAIFDTALILNDELYQEFDKTITKMNSNLLLYIMRREGFSWFINIVSNNNEFSHIKINKEFSSICSICRQLFKTENNIKLLTPYMRKYYEQML

SEQ ID NO: 45 - protein, 315 aa, Enterococcus faecalis
MYDSVVVNLGARCNASCEHCCFSCSPTKKEALDKNEVINLVENFSNNPKIKTISFTGGEIFLNYPFLYNLLKIVNSSGKISTLISNGFWGREIETVKKYFLDMNRMGVTNLSISHDDFHSKFIKTDYIRNILIESRKYPDIQITVNIAVSKNSTGDKIIHDLGEAILGIPVTKFPLIPVGEAKNINDDEFQNIYSLSHPNQLKCPGFEPVYHFNGNVYPCCSPAIFDTALILNDELYQEFDKTITKMNSNLLLYIMRREGFSWFINIVSNNNEFSHIKINKEFSSICSICRQLFKTENNIKLLTPYMRKYYEQML

SEQ ID NO: 46 - protein, 315 aa, Enterococcus faecalis
MYESVVVNLGARCNASCEHCCFSCSPTKKEALDKNEVINLVENFSNNPKIKTISFTGGEIFLNYPFLYSLLKIVNSSGKISTLISNGFWGREIETVKKYFLDMNRMGVTNLSISHDDFHSKFIKTDYIRNILIESRKYPDIQITVNIAVSKNSTGDKIIHDLGEAILGIPVTKFPLIPVGEAKNINDDEFQNIYSLSHPNQLKCPGFEPVYHFNGNVYPCCSPAIFDTALILNDELYQDFDKTITKMNSNLLLYIMRREGFSWFINIVSNNNEFSHIKINKEFSSICSICRQLFKTENNIKLLTPYMRKYYEQML

SEQ ID NO: 47 - protein, 322 aa, Enterococcus faecalis
MKEGVNLLYESVVVNLGARCNASCEHCCFSCSPTKKEALDKNEVINLVENFSNNPKIKTISFTGGEIFLNYPFLYSLLKIVNSSGKISTLISNGFWGREIETVKKYFLDMNRMGVTNLSISHDDFHSKFIKTDYIRNILIESRKYPDIQITVNIAVSKNSTGDKIIHDLGEAILGIPVTKFPLIPVGEAKNINDDEFQNIYSLSHPNQLKCPGFEPVYHFNGNVYPCCSPAIFDTALILNDELYQDFDKTITKMNSNLLLYIMRREGFSWFINIVSNNNEFSHIKINKEFSSICSICRQLFKTENNIKLLTPYMRKYYEQML

SEQ ID NO: 48 - protein, 322 aa, Enterococcus faecalis
MKEGVNLLYDSVVVNLGARCNASCEHCCFSCSPTKKEALDKNEVINLVENFSNNPKIKTISFTGGEIFLNYPFLYNLLKIVNSSGKISTLISNGFWGREIETVKKYFLDMNRMGVTNLSISHDDFHSKFIKTDYIRNILIESRKYPDIQITVNIAVSKNSTGDKIIHDLGEAILGIPVTKFPLIPVGEAKNINDDEFQNIYSLSHPNQLKCPGFEPVYHFNGNVYPCCSPAIFDTALILNDELYQEFDKTITKMNSNLLLYIMRREGFSWFINIVSNNNEFSHIKINKEFSSICSICRQLFKTENNIKLLTPYMRKYYEQML

SEQ ID NO: 49 - protein, 322 aa, Enterococcus faecalis
MKEGVNLLYESVVVNLGARCNASCEHCCFSCSPTKKEALDKNEVINLVENFSNNPKIKTISFTGGEIFLNYPFLYSLLKIVNSSGKISTLISNGFWGREIETVKKYFLDMNRMGVTNLSISHDDFHSKFIKTDYIRNILIESRKYPDIQITVNIAVSKNSTGDKIIHDLGEAILGIPVTKFPLIPVGEAKNINDDEFQNIYSLSHPNQLKCPGFEPVYHFNGNVYPCCSPAIFDTALILNDELYQYFDKTITKMNSNLLLYIMRREGFSWFINIVSNNNEFSHIKINKEFSSICSICRQLFKTENNIKLLTPYMRKYYEQML

SEQ ID NO: 50 - protein, 314 aa, Enterococcus faecalis
MYDSVVVNLGARCNASCEHCCFSCSPTKKEALDKNEVINLVENFSNNPKIKTISFTGGEIFLNYPFLYNLLKIVNSSGKISTLISNGFWGREIETVKKYFLDMNRMGVTNLSISHDDFHSKFIKTDYIRNILIESRKYPDIQITVNIAVSKNSTGDKIIHDLGEAILGIPVTKFPLIPVGEAKNINDDEFQNIYSLSHPNQLKCPGFEPVYHFNGNVYPCCSPAIFDTALILNDELYQEFDKTITKMNSNLLLYIMRREGFSWFINIVSNNNEFSHIKINKEFSSICSICRQLFKTENNIKLLTPYMSQVQTPV

SEQ ID NO: 51 - protein, 312 aa, Corynebacterium diphtheriae
MVALGIVIDRKCNIRCGHCCFSSTPQAEEHLTDEQILRIVKEGCETPAIDTISLSGGEALLRKPLVLEVLRVAKSYGKAATLVTNGFWGQNKKRAEETLFELKEAGLCALKISFDDFHQDLLKVEKVKNILDANLSVRVPIAINVAVSKNFSSDRILAALGESLMGVKVIKFPIQRVGAAEQYPEESIIRRHRIEDNLTCPGFEPTYHYDGKVYPCCSPTVFTTGLTFGKAEDLPVERAVSSIERNLLFAAIRQKGFKWLFERCIEERVLDISYIDRSYVDACEMCQILFSNPHTLKAVVSIVSNEYTSISK

SEQ ID NO: 52 - protein, 315 aa, Streptococcus agalactiae
MKSLVINLSQKCNAKCDHCCFSCLPNSVNCLTDEEIEAVVRYAETHEDVELVSLTGGEALLRKSKVLETIHRLSILGKDVTLITNGFWATNDKNTKSLLTSLRTAGLRYLTVSYDNYHSEYIPVDNIKRLFLHIKKFDIEVALNMVVDKKNRGVDLLDKLGESIFGVPITIVPASPVGRAKNLNMEDLYLKTIDELELTCPATGWEFVIHHDGYVYPCCSPSVFETNLRIGSIGDADISELEDKFYSNMLLYILKREGFTWFIDKMKLDLTGKKFVSSCEVCKFIFSDMNKIKSITDDIKEYYVKEFENIGVSKL

SEQ ID NO: 53 - protein, 316 aa, Bifidobacterium bohemicum
MTSICLTFSSKCNISCAHCCFSCGPHSEDHLSEEQSVKIVDDAIANAHVNSIGFSGGEALLHRNLLLSLMKRASEGNLKTTLVSNGFWGHSVANAQNILTLLKNAGLSTLTLSFDEFHEKFIPTQRIINILQANKYIGIPCHISMAVTKDHTGEELIHDLGEAGFTIPITRFPVVPVGAAAQLPKENIYSHYDANDPLICPGLQITYHFNGDVYPCCSPAVFHTCLSIGEVSNTPTHTALERVSRNKLFALMQRIGLRGIAEICKEHGIGPDLTKVPVVDPCDLCRKIFANSKTLEALLPYIDQAYRKTLPDKVQS

SEQ ID NO: 54 - protein, 27 aa, artificial sequence
  peptide
GLLDESQKLAKVNDLWYFVKSKENRWI

SEQ ID NO: 55 - protein, 19 aa, artificial sequence
  peptide
GLLDESQKLAKVNDLWYFV

SEQ ID NO: 56 - protein, 5 aa, artificial sequence
  peptide
LGSGH

SEQ ID NO: 57 - protein, 5 aa, artificial sequence
  segment
  MISC_FEATURE (3)..(3): X is any amino acid
WIXGS

SEQ ID NO: 58 - protein, 5 aa, artificial sequence
  segment
  MISC_FEATURE (3)..(3): X is any amino acid
WVXGS

SEQ ID NO: 59 - protein, 17 aa, artificial sequence
  peptide
  MISC_FEATURE (1)..(1): X is N or D
  MISC_FEATURE (7)..(7): X is V or I
  MISC_FEATURE (8)..(12): X is any amino acid
  MISC_FEATURE (14)..(14): X is V or I
  MISC_FEATURE (15)..(15): X is any amino acid
XDLWYFXXXXXXWXXGS

SEQ ID NO: 60 - protein, 18 aa, artificial sequence
  peptide
  MISC_FEATURE (1)..(1): X is N or D
  MISC_FEATURE (7)..(7): X is V or I
  MISC_FEATURE (8)..(13): X is any amino acid
  MISC_FEATURE (15)..(15): X is I or V
  MISC_FEATURE (16)..(16): X is any amino acid
XDLWYFXXXXXXXWXXGS

SEQ ID NO: 61 - protein, 17 aa, artificial sequence
  YydF33_49
WYFVKSKENRWILGSGH

SEQ ID NO: 62 - protein, 17 aa, artificial sequence
  Peptide-SA1
WYFVRSSKNRWVAGSAH

SEQ ID NO: 63 - protein, 17 aa, artificial sequence
  Peptide-SA2
WYFVRNSKNRWVAGSAH

SEQ ID NO: 64 - protein, 17 aa, artificial sequence
  Peptide-SE
WYFVKSKQNRWVVGSGH

SEQ ID NO: 65 - protein, 17 aa, artificial sequence
  Peptide-SP
WYFVKSQSNRWIVGSGH

SEQ ID NO: 66 - protein, 17 aa, artificial sequence
  YydF33_49AA
WYFAKSKENRWALGSGH

SEQ ID NO: 67 - protein, 17 aa, artificial sequence
  YydF33_49VV
WYFVKSKENRWVLGSGH

SEQ ID NO: 68 - protein, 17 aa, artificial sequence
  YydF33_49II
WYFIKSKENRWILGSGH

SEQ ID NO: 69 - protein, 5 aa, artificial sequence
  motif
  MISC_FEATURE (2)..(2): X is V, I or A
  MISC_FEATURE (3)..(3): X is any amino acid
WXXGS

SEQ ID NO: 70 - protein, 5 aa, artificial sequence
  motif
  MISC_FEATURE (3)..(3): X is any amino acid
WAXGS

SEQ ID NO: 71 - protein, 4 aa, artificial sequence
  motif
  MISC_FEATURE (4)..(4): X is V, I or A
WYFX

SEQ ID NO: 72 - protein, 17 aa, artificial sequence
  peptide
  MISC_FEATURE (4)..(4): X is V, I or A
  MISC_FEATURE (5)..(5): X is K or R
  MISC_FEATURE (6)..(8): X is a polar amino acid
  MISC_FEATURE (12)..(12): X is V, I or A
  MISC_FEATURE (13)..(13): X is an aliphatic amino acid
  MISC_FEATURE (16)..(16): X is any amino acid
WYFXXXXXNRWXXGSXH

SEQ ID NO: 73 - protein, 17 aa, artificial sequence
  peptide
  MISC_FEATURE (4)..(4): X is V, I or A
  MISC_FEATURE (5)..(5): X is R or K
  MISC_FEATURE (6)..(6): X is S or N
  MISC_FEATURE (7)..(7): X is S, Q or K
  MISC_FEATURE (8)..(8): X is E, K, S or Q
  MISC_FEATURE (12)..(12): X is V, I or A
  MISC_FEATURE (13)..(13): X is L, V or A
  MISC_FEATURE (16)..(16): X is A or G
WYFXXXXXNRWXXGSXH